European Patent Application EP 4 793 286 A1, published August 19, 2026. Title: ANTI-PD-1 MONOCLONAL ANTIBODY AND USE THEREOF. Applicant: SHANGHAI SCIZENG MEDICAL TECHNOLOGY CO., LTD. The sequence listing filed with the application follows.

SEQUENCE LISTING (55 sequences)

SEQ ID NO: 1 - protein, 5 aa, synthetic construct
  source 1..5: note = B1-1B5-H1L1/1B5-zu1-hIgG1/1B5-zu1-hIgG1 DD heavy chain variable region CDR1 amino acid sequence
NYPIE

SEQ ID NO: 2 - protein, 17 aa, synthetic construct
  source 1..17: note = B1-1B5-H1L1/1B5-zu1-hIgG1/1B5-zu1-hIgG1 DD heavy chain variable region CDR2 amino acid sequence
NFHPYNDDTKYNEKFKG

SEQ ID NO: 3 - protein, 11 aa, synthetic construct
  source 1..11: note = B1-1B5-H1L1/1B5-zu1-hIgG1/1B5-zu1-hIgG1 DD heavy chain variable region CDR3 amino acid sequence
EDYGTYGGFAY

SEQ ID NO: 4 - protein, 12 aa, synthetic construct
  source 1..12: note = B1-1B5-H1L1/1B5-zu1-hIgG1/1B5-zu1-hIgG1 DD light chain variable region CDR1 amino acid sequence
RASSSVSSSYLL

SEQ ID NO: 5 - protein, 7 aa, synthetic construct
  source 1..7: note = B1-1B5-H1L1/1B5-zu1-hIgG1/1B5-zu1-hIgG1 DD light chain variable region CDR2 amino acid sequence
STSNLAS

SEQ ID NO: 6 - protein, 9 aa, synthetic construct
  source 1..9: note = B1-1B5-H1L1/1B5-zu1-hIgG1/1B5-zu1-hIgG1 DD light chain variable region CDR3 amino acid sequence
QQYSGYPLT

SEQ ID NO: 7 - protein, 120 aa, synthetic construct
  source 1..120: note = B1-1B5-H1L1 heavy chain variable region amino acid sequence
EVQLQQSGAELVKPGASVKMSCKAFGYTFTNYPIEWMKQSHGKSLEWIGNFHPYNDDTKYNEKFKGKAKLTVEKSSSTVYLELSRLTSDDSAVYYCAREDYGTYGGFAYWGQGTLVTVSS

SEQ ID NO: 8 - protein, 108 aa, synthetic construct
  source 1..108: note = B1-1B5-H1L1 light chain variable region amino acid sequence
EITVTQSPAIMSASPGEKVTMTCRASSSVSSSYLLWYQQKSGASPKLWIYSTSNLASGVPARFSGSGSGTSYSLTISSVEAEDAATYYCQQYSGYPLTFGAGTKLELK

SEQ ID NO: 9 - DNA, 360 bp, synthetic construct
  source 1..360: mol_type = other DNA; note = B1-1B5-H1L1 heavy chain variable region nucleotide sequence
gaggtccagcttcagcagtctggggctgagctggtgaagcctggggcctcagtgaagatgtcctgcaaggcttttggctacaccttcactaactatccaatagagtggatgaagcagagtcatgggaagagcctagagtggattggaaattttcatccttacaatgatgatactaaatacaatgaaaaattcaagggcaaggccaaattgactgtagaaaaatcctctagcacagtctacttggagctcagccgattaacatctgatgactctgctgtttattactgtgcaagggaggactatggtacctacggggggtttgcttactggggccaagggactctggtcaccgtctcgagc

SEQ ID NO: 10 - DNA, 324 bp, synthetic construct
  source 1..324: mol_type = other DNA; note = B1-1B5-H1L1 light chain variable region nucleotide sequence
gaaataactgtgacccagtctccagcaatcatgtctgcatctccaggggaaaaggtcaccatgacctgcagggccagctcaagtgtaagttccagttacttgctctggtaccagcagaagtcaggtgcctcccccaaactctggatttatagcacatccaacttggcttctggagtccctgctcgcttcagtggcagtgggtctgggacctcttactctctcacaatcagcagtgtggaggctgaagatgctgccacttattactgccagcagtacagtggttacccactcacgttcggtgctgggaccaagctggagctgaaa

SEQ ID NO: 11 - protein, 450 aa, synthetic construct
  source 1..450: note = B1-1B5-H1L1 heavy chain amino acid sequence
EVQLQQSGAELVKPGASVKMSCKAFGYTFTNYPIEWMKQSHGKSLEWIGNFHPYNDDTKYNEKFKGKAKLTVEKSSSTVYLELSRLTSDDSAVYYCAREDYGTYGGFAYWGQGTLVTVSSASTKGPSVFPLAPSSKSTSGGTAALGCLVKDYFPEPVTVSWNSGALTSGVHTFPAVLQSSGLYSLSSVVTVPSSSLGTQTYICNVNHKPSNTKVDKKVEPKSCDKTHTCPPCPAPELLGGPSVFLFPPKPKDTLMISRTPEVTCVVVDVSHEDPEVKFNWYVDGVEVHNAKTKPREEQYNSTYRVVSVLTVLHQDWLNGKEYKCKVSNKALPAPIEKTISKAKGQPREPQVYTLPPSRDELTKNQVSLTCLVKGFYPSDIAVEWESNGQPENNYKTTPPVLDSDGSFFLYSKLTVDKSRWQQGNVFSCSVMHEALHNHYTQKSLSLSPGK

SEQ ID NO: 12 - protein, 215 aa, synthetic construct
  source 1..215: note = B1-1B5-H1L1 light chain amino acid sequence
EITVTQSPAIMSASPGEKVTMTCRASSSVSSSYLLWYQQKSGASPKLWIYSTSNLASGVPARFSGSGSGTSYSLTISSVEAEDAATYYCQQYSGYPLTFGAGTKLELKRTVAAPSVFIFPPSDEQLKSGTASVVCLLNNFYPREAKVQWKVDNALQSGNSQESVTEQDSKDSTYSLSSTLTLSKADYEKHKVYACEVTHQGLSSPVTKSFNRGEC

SEQ ID NO: 13 - DNA, 1350 bp, synthetic construct
  source 1..1350: mol_type = other DNA; note = B1-1B5-H1L1 heavy chain nucleotide sequence
gaggtccagcttcagcagtctggggctgagctggtgaagcctggggcctcagtgaagatgtcctgcaaggcttttggctacaccttcactaactatccaatagagtggatgaagcagagtcatgggaagagcctagagtggattggaaattttcatccttacaatgatgatactaaatacaatgaaaaattcaagggcaaggccaaattgactgtagaaaaatcctctagcacagtctacttggagctcagccgattaacatctgatgactctgctgtttattactgtgcaagggaggactatggtacctacggggggtttgcttactggggccaagggactctggtcaccgtctcgagcgctagcaccaagggcccatcggtcttccccctggcaccctcctccaagagcacctctgggggcacagcggccctgggctgcctggtcaaggactacttccccgaaccggtgacggtgtcgtggaactcaggcgccctgaccagcggcgtgcacaccttcccggctgtcctacagtcctcaggactctactccctcagcagcgtggtgaccgtgccctccagcagcttgggcacccagacctacatctgcaacgtgaatcacaagcccagcaacaccaaggtggacaagaaagttgagcccaaatcttgtgacaaaactcacacatgcccaccgtgcccagcacctgaactcctggggggaccgtcagtcttcctcttccccccaaaacccaaggacaccctcatgatctcccggacccctgaggtcacatgcgtggtggtggacgtgagccacgaagaccctgaggtcaagttcaactggtacgtggacggcgtggaggtgcataatgccaagacaaagccgcgggaggagcagtacaacagcacgtaccgtgtggtcagcgtcctcaccgtcctgcaccaggactggctgaatggcaaggagtacaagtgcaaggtctccaacaaagccctcccagcccccatcgagaaaaccatctccaaagccaaagggcagccccgagaaccacaggtgtacaccctgcctccatctcgggatgagctgaccaagaaccaggtcagcctgacctgcctggtcaaaggcttctatcccagcgacatcgccgtggagtgggagagcaatgggcagccggagaacaactacaagaccacgcctcccgtgctggactccgacggctccttcttcctctatagcaagctcaccgtggacaagagcaggtggcagcaggggaacgtcttctcatgctccgtgatgcatgaggctctgcacaaccactacacgcagaagagcctctccctgtctccgggtaaa

SEQ ID NO: 14 - DNA, 645 bp, synthetic construct
  source 1..645: mol_type = other DNA; note = B1-1B5-H1L1 light chain nucleotide sequence
gaaataactgtgacccagtctccagcaatcatgtctgcatctccaggggaaaaggtcaccatgacctgcagggccagctcaagtgtaagttccagttacttgctctggtaccagcagaagtcaggtgcctcccccaaactctggatttatagcacatccaacttggcttctggagtccctgctcgcttcagtggcagtgggtctgggacctcttactctctcacaatcagcagtgtggaggctgaagatgctgccacttattactgccagcagtacagtggttacccactcacgttcggtgctgggaccaagctggagctgaaacggaccgtggcggcgccatctgtcttcatcttcccgccatctgatgagcagttgaaatctggtaccgctagcgttgtgtgcctgctgaataacttctatcccagagaggccaaagtacagtggaaggtggataacgccctccaatcgggtaactcccaggagagtgtcacagagcaggacagcaaggacagcacctacagcctcagcagcaccctgacgctgagcaaagcagactacgagaaacacaaagtctacgcctgcgaagtcacccatcagggcctgagctcgcccgtcacaaagagcttcaacaggggagagtgt

SEQ ID NO: 15 - protein, 120 aa, synthetic construct
  source 1..120: note = 1B5-zu1-hIgG1/1B5-zu1-hIgG1 DD heavy chain variable region amino acid sequence
QVQLVQSGAEVKKPGASVKVSCKAFGYTFTNYPIEWMRQAPGQSLEWIGNFHPYNDDTKYNEKFKGRVTMTRDTSISTVYLELSRLRSDDTAVYYCAREDYGTYGGFAYWGQGTLVTVSS

SEQ ID NO: 16 - protein, 108 aa, synthetic construct
  source 1..108: note = 1B5-zu1-hIgG1/1B5-zu1-hIgG1 DD light chain variable region amino acid sequence
EIVLTQSPATLSLSPGERATLTCRASSSVSSSYLLWYQQKSGAAPRLWIYSTSNLASGVPARFSGSGSGTDFTLTISSLEPEDFATYYCQQYSGYPLTFGQGTKLEIK

SEQ ID NO: 17 - DNA, 360 bp, synthetic construct
  source 1..360: mol_type = other DNA; note = 1B5-zu1-hIgG1/1B5-zu1-hIgG1 DD heavy chain variable region nucleotide sequence
caggttcagctggttcagtctggcgccgaagtgaagaaacctggcgcctctgtgaaggtgtcctgcaaggctttcggctacacctttaccaactatcccatcgagtggatgcggcaggctcctggccaaagcctggaatggatcggcaactttcacccctacaacgacgacaccaagtacaacgagaagttcaagggccgcgtgaccatgaccagagacacctccatctccaccgtgtacctggaactgtcccggctgagatctgacgacaccgccgtgtactactgcgccagagaggattacggcacctacggcggctttgcttattggggccagggcacactggtcacagtgtcctct

SEQ ID NO: 18 - DNA, 324 bp, synthetic construct
  source 1..324: mol_type = other DNA; note = 1B5-zu1-hIgG1/1B5-zu1-hIgG1 DD light chain variable region nucleotide sequence
gagatcgtgctgacccagtctcctgccacactgtcactgtctccaggcgagagagctaccctgacctgcagagcctcttccagcgtgtcctcctcttacctgctgtggtatcagcagaagtccggcgctgctcccagactgtggatctactccacctccaatctggcctctggcgtgccagccagattttccggttctggctctggcaccgactttaccctgacaatctccagcctggaacctgaggacttcgccacctactactgccagcagtacagcggctaccctctgacctttggccagggcaccaagctggaaatcaag

SEQ ID NO: 19 - protein, 450 aa, synthetic construct
  source 1..450: note = 1B5-zu1-hIgG1 heavy chain amino acid sequence
QVQLVQSGAEVKKPGASVKVSCKAFGYTFTNYPIEWMRQAPGQSLEWIGNFHPYNDDTKYNEKFKGRVTMTRDTSISTVYLELSRLRSDDTAVYYCAREDYGTYGGFAYWGQGTLVTVSSASTKGPSVFPLAPSSKSTSGGTAALGCLVKDYFPEPVTVSWNSGALTSGVHTFPAVLQSSGLYSLSSVVTVPSSSLGTQTYICNVNHKPSNTKVDKKVEPKSCDKTHTCPPCPAPELLGGPSVFLFPPKPKDTLMISRTPEVTCVVVDVSHEDPEVKFNWYVDGVEVHNAKTKPREEQYNSTYRVVSVLTVLHQDWLNGKEYKCKVSNKALPAPIEKTISKAKGQPREPQVYTLPPSRDELTKNQVSLTCLVKGFYPSDIAVEWESNGQPENNYKTTPPVLDSDGSFFLYSKLTVDKSRWQQGNVFSCSVMHEALHNHYTQKSLSLSPGK

SEQ ID NO: 20 - protein, 215 aa, synthetic construct
  source 1..215: note = 1B5-zu1-hIgG1/1B5-zu1-hIgG1 DD light chain amino acid sequence
EIVLTQSPATLSLSPGERATLTCRASSSVSSSYLLWYQQKSGAAPRLWIYSTSNLASGVPARFSGSGSGTDFTLTISSLEPEDFATYYCQQYSGYPLTFGQGTKLEIKRTVAAPSVFIFPPSDEQLKSGTASVVCLLNNFYPREAKVQWKVDNALQSGNSQESVTEQDSKDSTYSLSSTLTLSKADYEKHKVYACEVTHQGLSSPVTKSFNRGEC

SEQ ID NO: 21 - DNA, 1350 bp, synthetic construct
  source 1..1350: mol_type = other DNA; note = 1B5-zu1-hIgG1 heavy chain nucleotide sequence
caggttcagctggttcagtctggcgccgaagtgaagaaacctggcgcctctgtgaaggtgtcctgcaaggctttcggctacacctttaccaactatcccatcgagtggatgcggcaggctcctggccaaagcctggaatggatcggcaactttcacccctacaacgacgacaccaagtacaacgagaagttcaagggccgcgtgaccatgaccagagacacctccatctccaccgtgtacctggaactgtcccggctgagatctgacgacaccgccgtgtactactgcgccagagaggattacggcacctacggcggctttgcttattggggccagggcacactggtcacagtgtcctctgcttccaccaagggcccctccgtgttccccctggctccctcttccaagagcaccagcggcggcaccgctgctctgggatgtctggtgaaggactacttccctgagcctgtgaccgtgtcctggaattccggcgccctgacctccggcgtgcacacattccctgctgtgctgcagtcctccggcctgtatagcctgtcctccgtggtgacagtgcctagctccagcctgggcacccagacctatatctgcaacgtgaaccacaagcctagcaataccaaggtggacaagaaggtggagcctaagagctgcgacaagacccacacctgtcctccatgtcctgctccagaactgctcggcggaccttccgtgttcctgtttcctccaaagcctaaggacaccctgatgatcagcagaacccctgaagtgacctgcgtggtggtggatgtgtcccacgaggatcccgaagtgaagttcaattggtacgtggacggcgtggaagtgcacaacgccaagaccaagcctagagaggaacagtacaacagcacctacagagtggtgtccgtgctgaccgtgctgcaccaggattggctgaacggcaaagagtacaagtgcaaggtgtccaacaaggccctgcctgctcctatcgagaaaaccatcagcaaggccaagggccagcctagggaaccccaggtttacacactgcctccaagcagggacgagctgaccaagaatcaggtgtccctgacctgcctggtcaagggcttctacccttccgatatcgccgtggaatgggagagcaatggccagcctgagaacaactacaagacaacccctcctgtgctggacagcgacggctcattcttcctgtacagcaagctgacagtggacaagagcagatggcagcagggcaacgtgttcagctgcagcgtgatgcacgaggccctgcacaaccactacacccagaagtccctgagcctgtctcctggcaaa

SEQ ID NO: 22 - DNA, 645 bp, synthetic construct
  source 1..645: mol_type = other DNA; note = 1B5-zu1-hIgG1/1B5-zu1-hIgG1 DD light chain nucleotide sequence
gagatcgtgctgacccagtctcctgccacactgtcactgtctccaggcgagagagctaccctgacctgcagagcctcttccagcgtgtcctcctcttacctgctgtggtatcagcagaagtccggcgctgctcccagactgtggatctactccacctccaatctggcctctggcgtgccagccagattttccggttctggctctggcaccgactttaccctgacaatctccagcctggaacctgaggacttcgccacctactactgccagcagtacagcggctaccctctgacctttggccagggcaccaagctggaaatcaagaggaccgtggctgcccccagcgtgttcatcttccctcctagcgacgagcagctgaagagcggcaccgctagcgtggtgtgtctgctgaataacttctatcccagggaggccaaggtgcagtggaaggtggataacgccctgcagagcggcaactcccaggagtccgtgaccgagcaggactccaaggacagcacctactccctgagctccaccctgaccctgtccaaggctgattatgagaagcacaaggtgtatgcttgcgaggtgacacaccagggcctgtccagccctgtgaccaagagcttcaaccggggcgagtgc

SEQ ID NO: 23 - protein, 450 aa, synthetic construct
  source 1..450: note = 1B5-zu1-hIgG1 DD heavy chain amino acid sequence
QVQLVQSGAEVKKPGASVKVSCKAFGYTFTNYPIEWMRQAPGQSLEWIGNFHPYNDDTKYNEKFKGRVTMTRDTSISTVYLELSRLRSDDTAVYYCAREDYGTYGGFAYWGQGTLVTVSSASTKGPSVFPLAPSSKSTSGGTAALGCLVKDYFPEPVTVSWNSGALTSGVHTFPAVLQSSGLYSLSSVVTVPSSSLGTQTYICNVNHKPSNTKVDKKVEPKSCDKTHTCPPCPAPELLGGPDVFLFPPKPKDTLMISRTPEVTCVVVDVSDEDPEVKFNWYVDGVEVHNAKTKPREEQYNSTYRVVSVLTVLHQDWLNGKEYKCKVSNKALPAPIEKTISKAKGQPREPQVYTLPPSRDELTKNQVSLTCLVKGFYPSDIAVEWESNGQPENNYKTTPPVLDSDGSFFLYSKLTVDKSRWQQGNVFSCSVMHEALHNHYTQKSLSLSPGK

SEQ ID NO: 24 - DNA, 1350 bp, synthetic construct
  source 1..1350: mol_type = other DNA; note = 1B5-zu1-hIgG1 DD heavy chain nucleotide sequence
caggttcagctggttcagtctggcgccgaagtgaagaaacctggcgcctctgtgaaggtgtcctgcaaggctttcggctacacctttaccaactatcccatcgagtggatgcggcaggctcctggccaaagcctggaatggatcggcaactttcacccctacaacgacgacaccaagtacaacgagaagttcaagggccgcgtgaccatgaccagagacacctccatctccaccgtgtacctggaactgtcccggctgagatctgacgacaccgccgtgtactactgcgccagagaggattacggcacctacggcggctttgcttattggggccagggcacactggtcacagtgtcctctgctagcaccaagggcccatcggtcttccccctggcaccctcctccaagagcacctctgggggcacagcggccctgggctgcctggtcaaggactacttccccgaaccggtgacggtgtcgtggaactcaggcgccctgaccagcggcgtgcacaccttcccggctgtcctacagtcctcaggactctactccctcagcagcgtggtgaccgtgccctccagcagcttgggcacccagacctacatctgcaacgtgaatcacaagcccagcaacaccaaggtggacaagaaagttgagcccaaatcttgtgacaaaactcacacatgcccaccgtgcccagcacctgaactcctggggggaccggacgtcttcctcttccccccaaaacccaaggacaccctcatgatctcccggacccctgaggtcacatgcgtggtggtggacgtgagcgacgaagaccctgaggtcaagttcaactggtacgtggacggcgtggaggtgcataatgccaagacaaagccgcgggaggagcagtacaacagcacgtaccgtgtggtcagcgtcctcaccgtcctgcaccaggactggctgaatggcaaggagtacaagtgcaaggtctccaacaaagccctcccagcccccatcgagaaaaccatctccaaagccaaagggcagccccgagaaccacaggtgtacaccctgcctccatctcgggatgagctgaccaagaaccaggtcagcctgacctgcctggtcaaaggcttctatcccagcgacatcgccgtggagtgggagagcaatgggcagccggagaacaactacaagaccacgcctcccgtgctggactccgacggctccttcttcctctatagcaagctcaccgtggacaagagcaggtggcagcaggggaacgtcttctcatgctccgtgatgcatgaggctctgcacaaccactacacgcagaagagcctctccctgtctccgggtaaa

SEQ ID NO: 25 - protein, 5 aa, synthetic construct
  source 1..5: note = B1-1C4-H1L1/1C4-zu1-hIgG1/1C4-zu1-hIgG1 DD heavy chain variable region CDR1 amino acid sequence
SYWIT

SEQ ID NO: 26 - protein, 17 aa, synthetic construct
  source 1..17: note = B1-1C4-H1L1/1C4-zu1-hIgG1/1C4-zu1-hIgG1 DD heavy chain variable region CDR2 amino acid sequence
RIAPGSGSIYYDEMFKD

SEQ ID NO: 27 - protein, 10 aa, synthetic construct
  source 1..10: note = B1-1C4-H1L1/1C4-zu1-hIgG1/1C4-zu1-hIgG1 DD heavy chain variable region CDR3 amino acid sequence
LGNYGWTMDY

SEQ ID NO: 28 - protein, 11 aa, synthetic construct
  source 1..11: note = B1-1C4-H1L1/1C4-zu1-hIgG1/1C4-zu1-hIgG1 DD light chain variable region CDR1 amino acid sequence
KASQSVTNNVA

SEQ ID NO: 29 - protein, 7 aa, synthetic construct
  source 1..7: note = B1-1C4-H1L1/1C4-zu1-hIgG1/1C4-zu1-hIgG1 DD light chain variable region CDR2 amino acid sequence
YVSNRYT

SEQ ID NO: 30 - protein, 8 aa, synthetic construct
  source 1..8: note = B1-1C4-H1L1/1C4-zu1-hIgG1/1C4-zu1-hIgG1 DD light chain variable region CDR3 amino acid sequence
QQDYSSWT

SEQ ID NO: 31 - protein, 119 aa, synthetic construct
  source 1..119: note = B1-1C4-H1L1 heavy chain variable region amino acid sequence
EVQLQQSGDDLVKPGASVKLSCKASGYTFTSYWITWIKQRPGQGLEWIGRIAPGSGSIYYDEMFKDKATLTVDPSSSTAYIQLSSLSSEDSAVYFCARLGNYGWTMDYWGQGTSVTVSS

SEQ ID NO: 32 - protein, 106 aa, synthetic construct
  source 1..106: note = B1-1C4-H1L1 light chain variable region amino acid sequence
DIVMTQTPKFLLVSAGDRVTITCKASQSVTNNVAWYQQAPGQSPKLLIYYVSNRYTGVPDRFAGSGYGTDFTFTISTVQAEDLAVYFCQQDYSSWTFGGGTKLEIK

SEQ ID NO: 33 - DNA, 357 bp, synthetic construct
  source 1..357: mol_type = other DNA; note = B1-1C4-H1L1 heavy chain variable region nucleotide sequence
gaggtccagcttcagcagtctggagatgatctggtaaagcctggggcctcagtgaagctgtcctgcaaggcttctggctacaccttcaccagctactggattacctggataaaacagaggcctggacagggccttgagtggataggacgtattgctcctggaagtggtagtatttactacgatgaaatgttcaaggacaaggcaacactgactgtagacccatcctccagcacagcctacattcaactcagcagcctgtcatctgaggactctgctgtctatttctgtgcaagattgggtaactacggatggactatggactactggggtcaaggaacctcagtcaccgtctcgagc

SEQ ID NO: 34 - DNA, 318 bp, synthetic construct
  source 1..318: mol_type = other DNA; note = B1-1C4-H1L1 light chain variable region nucleotide sequence
gatattgtgatgacccagactcccaaattcctgcttgtatcagcaggagacagggttaccataacctgcaaggccagtcagagtgtgactaataatgtagcttggtatcaacaggcgccaggtcagtctcctaaactgctgatatattatgtatccaatcgctacactggagtccctgatcgcttcgctggcagtggatatgggacggatttcactttcaccatcagcactgtgcaggctgaagacctggcagtttatttctgtcaacaggattatagctcttggacgttcggtgggggcaccaagctggaaatcaaa

SEQ ID NO: 35 - protein, 449 aa, synthetic construct
  source 1..449: note = B1-1C4-H1L1 heavy chain amino acid sequence
EVQLQQSGDDLVKPGASVKLSCKASGYTFTSYWITWIKQRPGQGLEWIGRIAPGSGSIYYDEMFKDKATLTVDPSSSTAYIQLSSLSSEDSAVYFCARLGNYGWTMDYWGQGTSVTVSSASTKGPSVFPLAPSSKSTSGGTAALGCLVKDYFPEPVTVSWNSGALTSGVHTFPAVLQSSGLYSLSSVVTVPSSSLGTQTYICNVNHKPSNTKVDKKVEPKSCDKTHTCPPCPAPELLGGPSVFLFPPKPKDTLMISRTPEVTCVVVDVSHEDPEVKFNWYVDGVEVHNAKTKPREEQYNSTYRVVSVLTVLHQDWLNGKEYKCKVSNKALPAPIEKTISKAKGQPREPQVYTLPPSRDELTKNQVSLTCLVKGFYPSDIAVEWESNGQPENNYKTTPPVLDSDGSFFLYSKLTVDKSRWQQGNVFSCSVMHEALHNHYTQKSLSLSPGK

SEQ ID NO: 36 - protein, 213 aa, synthetic construct
  source 1..213: note = B1-1C4-H1L1 light chain amino acid sequence
DIVMTQTPKFLLVSAGDRVTITCKASQSVTNNVAWYQQAPGQSPKLLIYYVSNRYTGVPDRFAGSGYGTDFTFTISTVQAEDLAVYFCQQDYSSWTFGGGTKLEIKRTVAAPSVFIFPPSDEQLKSGTASVVCLLNNFYPREAKVQWKVDNALQSGNSQESVTEQDSKDSTYSLSSTLTLSKADYEKHKVYACEVTHQGLSSPVTKSFNRGEC

SEQ ID NO: 37 - DNA, 1347 bp, synthetic construct
  source 1..1347: mol_type = other DNA; note = B1-1C4-H1L1 heavy chain nucleotide sequence
gaggtccagcttcagcagtctggagatgatctggtaaagcctggggcctcagtgaagctgtcctgcaaggcttctggctacaccttcaccagctactggattacctggataaaacagaggcctggacagggccttgagtggataggacgtattgctcctggaagtggtagtatttactacgatgaaatgttcaaggacaaggcaacactgactgtagacccatcctccagcacagcctacattcaactcagcagcctgtcatctgaggactctgctgtctatttctgtgcaagattgggtaactacggatggactatggactactggggtcaaggaacctcagtcaccgtctcgagcgctagcaccaagggcccatcggtcttccccctggcaccctcctccaagagcacctctgggggcacagcggccctgggctgcctggtcaaggactacttccccgaaccggtgacggtgtcgtggaactcaggcgccctgaccagcggcgtgcacaccttcccggctgtcctacagtcctcaggactctactccctcagcagcgtggtgaccgtgccctccagcagcttgggcacccagacctacatctgcaacgtgaatcacaagcccagcaacaccaaggtggacaagaaagttgagcccaaatcttgtgacaaaactcacacatgcccaccgtgcccagcacctgaactcctggggggaccgtcagtcttcctcttccccccaaaacccaaggacaccctcatgatctcccggacccctgaggtcacatgcgtggtggtggacgtgagccacgaagaccctgaggtcaagttcaactggtacgtggacggcgtggaggtgcataatgccaagacaaagccgcgggaggagcagtacaacagcacgtaccgtgtggtcagcgtcctcaccgtcctgcaccaggactggctgaatggcaaggagtacaagtgcaaggtctccaacaaagccctcccagcccccatcgagaaaaccatctccaaagccaaagggcagccccgagaaccacaggtgtacaccctgcctccatctcgggatgagctgaccaagaaccaggtcagcctgacctgcctggtcaaaggcttctatcccagcgacatcgccgtggagtgggagagcaatgggcagccggagaacaactacaagaccacgcctcccgtgctggactccgacggctccttcttcctctatagcaagctcaccgtggacaagagcaggtggcagcaggggaacgtcttctcatgctccgtgatgcatgaggctctgcacaaccactacacgcagaagagcctctccctgtctccgggtaaa

SEQ ID NO: 38 - DNA, 639 bp, synthetic construct
  source 1..639: mol_type = other DNA; note = B1-1C4-H1L1 light chain nucleotide sequence
gatattgtgatgacccagactcccaaattcctgcttgtatcagcaggagacagggttaccataacctgcaaggccagtcagagtgtgactaataatgtagcttggtatcaacaggcgccaggtcagtctcctaaactgctgatatattatgtatccaatcgctacactggagtccctgatcgcttcgctggcagtggatatgggacggatttcactttcaccatcagcactgtgcaggctgaagacctggcagtttatttctgtcaacaggattatagctcttggacgttcggtgggggcaccaagctggaaatcaaacggaccgtggcggcgccatctgtcttcatcttcccgccatctgatgagcagttgaaatctggtaccgctagcgttgtgtgcctgctgaataacttctatcccagagaggccaaagtacagtggaaggtggataacgccctccaatcgggtaactcccaggagagtgtcacagagcaggacagcaaggacagcacctacagcctcagcagcaccctgacgctgagcaaagcagactacgagaaacacaaagtctacgcctgcgaagtcacccatcagggcctgagctcgcccgtcacaaagagcttcaacaggggagagtgt

SEQ ID NO: 39 - protein, 119 aa, synthetic construct
  source 1..119: note = 1C4-zu1-hIgG1/1C4-zu1-hIgG1 DD heavy chain variable region amino acid sequence
QVQLVQSGAEVKKPGASVKVSCKASGYTFTSYWITWIRQAPGQGLEWIGRIAPGSGSIYYDEMFKDRVTMTVDPSTSTAYIELSSLRSEDTAVYYCARLGNYGWTMDYWGQGTTVTVSS

SEQ ID NO: 40 - protein, 106 aa, synthetic construct
  source 1..106: note = 1C4-zu1-hIgG1/1C4-zu1-hIgG1 DD light chain variable region amino acid sequence
DIVMTQSPKSLAVSLGERATINCKASQSVTNNVAWYQQKPGQPPKLLIYYVSNRYTGVPDRFSGSGYGTDFTLTISSLQAEDVAVYFCQQDYSSWTFGGGTKVEIK

SEQ ID NO: 41 - DNA, 357 bp, synthetic construct
  source 1..357: mol_type = other DNA; note = 1C4-zu1-hIgG1/1C4-zu1-hIgG1 DD heavy chain variable region nucleotide sequence
caggttcagctggttcagtctggcgccgaagtgaagaaacctggcgcctctgtgaaggtgtcctgcaaggcttccggctacacctttaccagctactggatcacctggatcagacaggctcccggccaaggcctggaatggatcggaagaatcgctcctggctccggctccatctactacgacgagatgttcaaggaccgcgtgaccatgacagtggacccttctacctccaccgcctacatcgagctgtccagcctgagatctgaggacaccgccgtgtactactgtgccagactgggcaactacggctggacaatggattactggggccagggcaccaccgtgacagtctcttct

SEQ ID NO: 42 - DNA, 318 bp, synthetic construct
  source 1..318: mol_type = other DNA; note = 1C4-zu1-hIgG1/1C4-zu1-hIgG1 DD light chain variable region nucleotide sequence
gacatcgtgatgacccagtctccaaagtctctggccgtgtctctgggcgagagagccaccatcaattgcaaggcctctcagtccgtgaccaacaacgtggcctggtatcagcagaagcctggccagcctcctaagctgctgatctactacgtgtccaaccggtacaccggcgtgcccgatagattttccggctctggctacggcaccgactttaccctgacaatcagctccctgcaggccgaggatgtggccgtgtacttctgccagcaagactactcctcctggacctttggcggaggcaccaaggtggaaatcaag

SEQ ID NO: 43 - protein, 449 aa, synthetic construct
  source 1..449: note = 1C4-zu1-hIgG1 heavy chain amino acid sequence
QVQLVQSGAEVKKPGASVKVSCKASGYTFTSYWITWIRQAPGQGLEWIGRIAPGSGSIYYDEMFKDRVTMTVDPSTSTAYIELSSLRSEDTAVYYCARLGNYGWTMDYWGQGTTVTVSSASTKGPSVFPLAPSSKSTSGGTAALGCLVKDYFPEPVTVSWNSGALTSGVHTFPAVLQSSGLYSLSSVVTVPSSSLGTQTYICNVNHKPSNTKVDKKVEPKSCDKTHTCPPCPAPELLGGPSVFLFPPKPKDTLMISRTPEVTCVVVDVSHEDPEVKFNWYVDGVEVHNAKTKPREEQYNSTYRVVSVLTVLHQDWLNGKEYKCKVSNKALPAPIEKTISKAKGQPREPQVYTLPPSRDELTKNQVSLTCLVKGFYPSDIAVEWESNGQPENNYKTTPPVLDSDGSFFLYSKLTVDKSRWQQGNVFSCSVMHEALHNHYTQKSLSLSPGK

SEQ ID NO: 44 - protein, 213 aa, synthetic construct
  source 1..213: note = 1C4-zu1-hIgG1/1C4-zu1-hIgG1 DD light chain amino acid sequence
DIVMTQSPKSLAVSLGERATINCKASQSVTNNVAWYQQKPGQPPKLLIYYVSNRYTGVPDRFSGSGYGTDFTLTISSLQAEDVAVYFCQQDYSSWTFGGGTKVEIKRTVAAPSVFIFPPSDEQLKSGTASVVCLLNNFYPREAKVQWKVDNALQSGNSQESVTEQDSKDSTYSLSSTLTLSKADYEKHKVYACEVTHQGLSSPVTKSFNRGEC

SEQ ID NO: 45 - DNA, 1347 bp, synthetic construct
  source 1..1347: mol_type = other DNA; note = 1C4-zu1-hIgG1 heavy chain nucleotide sequence
caggttcagctggttcagtctggcgccgaagtgaagaaacctggcgcctctgtgaaggtgtcctgcaaggcttccggctacacctttaccagctactggatcacctggatcagacaggctcccggccaaggcctggaatggatcggaagaatcgctcctggctccggctccatctactacgacgagatgttcaaggaccgcgtgaccatgacagtggacccttctacctccaccgcctacatcgagctgtccagcctgagatctgaggacaccgccgtgtactactgtgccagactgggcaactacggctggacaatggattactggggccagggcaccaccgtgacagtctcttctgcttccaccaagggcccctccgtgttccccctggctccctcttccaagagcaccagcggcggcaccgctgctctgggatgtctggtgaaggactacttccctgagcctgtgaccgtgtcctggaattccggcgccctgacctccggcgtgcacacattccctgctgtgctgcagtcctccggcctgtatagcctgtcctccgtggtgacagtgcctagctccagcctgggcacccagacctatatctgcaacgtgaaccacaagcctagcaataccaaggtggacaagaaggtggagcctaagagctgcgacaagacccacacctgtcctccatgtcctgctccagaactgctcggcggaccttccgtgttcctgtttcctccaaagcctaaggacaccctgatgatcagcagaacccctgaagtgacctgcgtggtggtggatgtgtcccacgaggatcccgaagtgaagttcaattggtacgtggacggcgtggaagtgcacaacgccaagaccaagcctagagaggaacagtacaacagcacctacagagtggtgtccgtgctgaccgtgctgcaccaggattggctgaacggcaaagagtacaagtgcaaggtgtccaacaaggccctgcctgctcctatcgagaaaaccatcagcaaggccaagggccagcctagggaaccccaggtttacacactgcctccaagcagggacgagctgaccaagaatcaggtgtccctgacctgcctggtcaagggcttctacccttccgatatcgccgtggaatgggagagcaatggccagcctgagaacaactacaagacaacccctcctgtgctggacagcgacggctcattcttcctgtacagcaagctgacagtggacaagagcagatggcagcagggcaacgtgttcagctgcagcgtgatgcacgaggccctgcacaaccactacacccagaagtccctgagcctgtctcctggcaaa

SEQ ID NO: 46 - DNA, 639 bp, synthetic construct
  source 1..639: mol_type = other DNA; note = 1C4-zu1-hIgG1/1C4-zu1-hIgG1 DD light chain nucleotide sequence
gacatcgtgatgacccagtctccaaagtctctggccgtgtctctgggcgagagagccaccatcaattgcaaggcctctcagtccgtgaccaacaacgtggcctggtatcagcagaagcctggccagcctcctaagctgctgatctactacgtgtccaaccggtacaccggcgtgcccgatagattttccggctctggctacggcaccgactttaccctgacaatcagctccctgcaggccgaggatgtggccgtgtacttctgccagcaagactactcctcctggacctttggcggaggcaccaaggtggaaatcaagaggaccgtggctgcccccagcgtgttcatcttccctcctagcgacgagcagctgaagagcggcaccgctagcgtggtgtgtctgctgaataacttctatcccagggaggccaaggtgcagtggaaggtggataacgccctgcagagcggcaactcccaggagtccgtgaccgagcaggactccaaggacagcacctactccctgagctccaccctgaccctgtccaaggctgattatgagaagcacaaggtgtatgcttgcgaggtgacacaccagggcctgtccagccctgtgaccaagagcttcaaccggggcgagtgc

SEQ ID NO: 47 - protein, 449 aa, synthetic construct
  source 1..449: note = 1C4-zu1-hIgG1 DD heavy chain amino acid sequence
QVQLVQSGAEVKKPGASVKVSCKASGYTFTSYWITWIRQAPGQGLEWIGRIAPGSGSIYYDEMFKDRVTMTVDPSTSTAYIELSSLRSEDTAVYYCARLGNYGWTMDYWGQGTTVTVSSASTKGPSVFPLAPSSKSTSGGTAALGCLVKDYFPEPVTVSWNSGALTSGVHTFPAVLQSSGLYSLSSVVTVPSSSLGTQTYICNVNHKPSNTKVDKKVEPKSCDKTHTCPPCPAPELLGGPDVFLFPPKPKDTLMISRTPEVTCVVVDVSDEDPEVKFNWYVDGVEVHNAKTKPREEQYNSTYRVVSVLTVLHQDWLNGKEYKCKVSNKALPAPIEKTISKAKGQPREPQVYTLPPSRDELTKNQVSLTCLVKGFYPSDIAVEWESNGQPENNYKTTPPVLDSDGSFFLYSKLTVDKSRWQQGNVFSCSVMHEALHNHYTQKSLSLSPGK

SEQ ID NO: 48 - DNA, 1347 bp, synthetic construct
  source 1..1347: mol_type = other DNA; note = 1C4-zu1-hIgG1 DD heavy chain nucleotide sequence
caggttcagctggttcagtctggcgccgaagtgaagaaacctggcgcctctgtgaaggtgtcctgcaaggcttccggctacacctttaccagctactggatcacctggatcagacaggctcccggccaaggcctggaatggatcggaagaatcgctcctggctccggctccatctactacgacgagatgttcaaggaccgcgtgaccatgacagtggacccttctacctccaccgcctacatcgagctgtccagcctgagatctgaggacaccgccgtgtactactgtgccagactgggcaactacggctggacaatggattactggggccagggcaccaccgtgacagtctcttctgctagcaccaagggcccatcggtcttccccctggcaccctcctccaagagcacctctgggggcacagcggccctgggctgcctggtcaaggactacttccccgaaccggtgacggtgtcgtggaactcaggcgccctgaccagcggcgtgcacaccttcccggctgtcctacagtcctcaggactctactccctcagcagcgtggtgaccgtgccctccagcagcttgggcacccagacctacatctgcaacgtgaatcacaagcccagcaacaccaaggtggacaagaaagttgagcccaaatcttgtgacaaaactcacacatgcccaccgtgcccagcacctgaactcctggggggaccggacgtcttcctcttccccccaaaacccaaggacaccctcatgatctcccggacccctgaggtcacatgcgtggtggtggacgtgagcgacgaagaccctgaggtcaagttcaactggtacgtggacggcgtggaggtgcataatgccaagacaaagccgcgggaggagcagtacaacagcacgtaccgtgtggtcagcgtcctcaccgtcctgcaccaggactggctgaatggcaaggagtacaagtgcaaggtctccaacaaagccctcccagcccccatcgagaaaaccatctccaaagccaaagggcagccccgagaaccacaggtgtacaccctgcctccatctcgggatgagctgaccaagaaccaggtcagcctgacctgcctggtcaaaggcttctatcccagcgacatcgccgtggagtgggagagcaatgggcagccggagaacaactacaagaccacgcctcccgtgctggactccgacggctccttcttcctctatagcaagctcaccgtggacaagagcaggtggcagcaggggaacgtcttctcatgctccgtgatgcatgaggctctgcacaaccactacacgcagaagagcctctccctgtctccgggtaaa

SEQ ID NO: 49 - protein, 288 aa, synthetic construct
  source 1..288: note = Full-length hPD-1 amino acid sequence
MQIPQAPWPVVWAVLQLGWRPGWFLDSPDRPWNPPTFSPALLVVTEGDNATFTCSFSNTSESFVLNWYRMSPSNQTDKLAAFPEDRSQPGQDCRFRVTQLPNGRDFHMSVVRARRNDSGTYLCGAISLAPKAQIKESLRAELRVTERRAEVPTAHPSPSPRPAGQFQTLVVGVVGGLLGSLVLLVWVLAVICSRAARGTIGARRTGQPLKEDPSAVPVFSVDYGELDFQWREKTPEPPVPCVPEQTEYATIVFPSGMGTSSPARRGSADGPRSAQPLRPEDGHCSWPL

SEQ ID NO: 50 - protein, 147 aa, synthetic construct
  source 1..147: note = hPD-1 ECD amino acid sequence
FLDSPDRPWNPPTFSPALLVVTEGDNATFTCSFSNTSESFVLNWYRMSPSNQTDKLAAFPEDRSQPGQDCRFRVTQLPNGRDFHMSVVRARRNDSGTYLCGAISLAPKAQIKESLRAELRVTERRAEVPTAHPSPSPRPAGQFQTLV

SEQ ID NO: 51 - protein, 330 aa, synthetic construct [sequence omitted]

SEQ ID NO: 52 - protein, 330 aa, synthetic construct
  source 1..330: note = hIgG1(DD) heavy chain constant region amino acid sequence
ASTKGPSVFPLAPSSKSTSGGTAALGCLVKDYFPEPVTVSWNSGALTSGVHTFPAVLQSSGLYSLSSVVTVPSSSLGTQTYICNVNHKPSNTKVDKKVEPKSCDKTHTCPPCPAPELLGGPDVFLFPPKPKDTLMISRTPEVTCVVVDVSDEDPEVKFNWYVDGVEVHNAKTKPREEQYNSTYRVVSVLTVLHQDWLNGKEYKCKVSNKALPAPIEKTISKAKGQPREPQVYTLPPSRDELTKNQVSLTCLVKGFYPSDIAVEWESNGQPENNYKTTPPVLDSDGSFFLYSKLTVDKSRWQQGNVFSCSVMHEALHNHYTQKSLSLSPGK

SEQ ID NO: 53 - protein, 107 aa, synthetic construct [sequence omitted]

SEQ ID NO: 54 - protein, 288 aa, synthetic construct
  source 1..288: note = cPD-1 amino acid sequence
MQIPQAPWPVVWAVLQLGWRPGWFLESPDRPWNAPTFSPALLLVTEGDNATFTCSFSNASESFVLNWYRMSPSNQTDKLAAFPEDRSQPGQDCRFRVTRLPNGRDFHMSVVRARRNDSGTYLCGAISLAPKAQIKESLRAELRVTERRAEVPTAHPSPSPRPAGQFQALVVGVVGGLLGSLVLLVWVLAVICSRAAQGTIEARRTGQPLKEDPSAVPVFSVDYGELDFQWREKTPEPPAPCVPEQTEYATIVFPSGLGTSSPARRGSADGPRSPRPLRPEDGHCSWPL

SEQ ID NO: 55 - protein, 147 aa, synthetic construct
  source 1..147: note = cPD-1 ECD amino acid sequence
FLESPDRPWNAPTFSPALLLVTEGDNATFTCSFSNASESFVLNWYRMSPSNQTDKLAAFPEDRSQPGQDCRFRVTRLPNGRDFHMSVVRARRNDSGTYLCGAISLAPKAQIKESLRAELRVTERRAEVPTAHPSPSPRPAGQFQALV